European Patent Application EP 4 487 857 A1, published January 8, 2025. Title: Treatment agent for demyelinating disease and peripheral neuropathy. Applicant: Cysay Inc. The sequence listing filed with the application follows.

SEQUENCE LISTING (26 sequences)

SEQ ID NO: 1 - DNA, 2223 bp, synthetic construct
  misc_feature 1..2223: note = DNA fragment for gene transduction
  misc_feature 1..2223: note = SYN4122-4-4
  source 1..2223: mol_type = other DNA
acgctgttttgacctccatagaagacaccgactctactagaggatctatttccggtgaattcgccacccaccaaaagagaactgcaatgtttcaggacccacaggagcgacccagaaagttaccacagttatgcacagagctgcaaacaactatacatgatataatattagaatgtgtgtactgcaagcaacagttactgcgacgtgaggtatatgactttgcttttcgggatttatgcatagtatatagagatgggaatccatatgctgtatgtgataaatgtttaaagttttattctaaaattagtgagtatagacattattgttatagtttgtatggaacaacattagaacagcaatacaacaaaccgttgtgtgatttgttaattaggtgtattaactgtcaaaagccactgtgtcctgaagaaaagcaaagacatctggacaaaaagcaaagattccataatataaggggtcggtggaccggtcgatgtatgtcttgttgcagatcatcaagaacacgtagagaaacccagctgggatctgaaggcagaggctctctgctgacatgtggggatgtggaggaaaatcctggccctacgcgtcatggagatacacctacattgcatgaatatatgttagatttgcaaccagagacaactgatctctactgttatgagcaattaaatgacagctcagaggaggaggatgaaatagatggtccagctggacaagcagaaccggacagagcccattacaatattgtaaccttttgttgcaagtgtgactctacgcttcggttgtgcgtacaaagcacacacgtagacattcgtactttggaagacctgttaatgggcacactaggaattgtgtgccccatctgttctcagaaaccaggatctgaaggtaggggaagtttgcttacttgcggtgacgtcgaagagaatccaggaccagatggccgcaacatgccgcgcgctccccgctgccgagccgtgcgctccctgctgcgcagccactaccgcgaggtgctgccgctggccacgttcgtgcggcgcctggggccccagggctggcggctggtgcagcgcggggacccggcggctttccgcgcgctggtggcccagtgcctggtgtgcgtgccctgggacgcacggccgccccccgccgccccctccttccgccaggtgtcctgcctgaaggagctggtggcccgagtgctgcagaggctgtgcgagcgcggcgcgaagaacgtgctggccttcggcttcgcgctgctggacggggcccgcgggggcccccccgaggccttcaccaccagcgtgcgcagctacctgcccaacacggtgaccgacgcactgcgggggagcggggcgtgggggctgctgctgcgccgcgtgggcgacgacgtgctggttcacctgctggcacgctgcgcgctctttgtgctggtggctcccagctgcgcctaccaggtgtgcgggccgccgctgtaccagctcggcgctgccactcaggcccggcccccgccacacgctagtggaccccgaaggcgtctgggatgcgaacgggcctggaaccatagcgtcagggaggccggggtccccctgggcctgccagccccgggtgcgaggaggcgcgggggcagtgccagccgaagtctgccgttgcccaagaggcccaggcgtggcgctgcccctgagccggagcggacgcccgttgggcaggggtcctgggcccacccgggcaggacgcgtggaccgagtgaccgtggtttctgtgtggtgtcacctgccagacccgccgaagaagccacctctttggagggtgcgctctctggcacgcgccactcccacccatccgtgggccgccagcaccacgcgggccccccatccacatcgcggccaccacgtccctgggacacgccttgtcccccggtgtacgccgagaccaagcacttcctctactcctcaggcgacaaggagcagctgcggccctccttcctactcagctctctgaggcccagcctgactggcgctcggaggctcgtggagaccatctttctgggttccaggccctggatgccagggactccccgcaggttgccccgcctgccccagcgctactggcaaatgcggcccctgtttctggagctgcttgggaaccacgcgcagtgcccctacggggtgctcctcaagacgcactgcccgctgcgagctgcgg

SEQ ID NO: 2 - DNA, 3399 bp, Homo sapiens
  misc_feature 1..3399: note = hTERT
  gene 1..3399: note = hTERT
  source 1..3399: mol_type = genomic DNA
atgccgcgcgctccccgctgccgagccgtgcgctccctgctgcgcagccactaccgcgaggtgctgccgctggccacgttcgtgcggcgcctggggccccagggctggcggctggtgcagcgcggggacccggcggctttccgcgcgctggtggcccagtgcctggtgtgcgtgccctgggacgcacggccgccccccgccgccccctccttccgccaggtgtcctgcctgaaggagctggtggcccgagtgctgcagaggctgtgcgagcgcggcgcgaagaacgtgctggccttcggcttcgcgctgctggacggggcccgcgggggcccccccgaggccttcaccaccagcgtgcgcagctacctgcccaacacggtgaccgacgcactgcgggggagcggggcgtgggggctgctgctgcgccgcgtgggcgacgacgtgctggttcacctgctggcacgctgcgcgctctttgtgctggtggctcccagctgcgcctaccaggtgtgcgggccgccgctgtaccagctcggcgctgccactcaggcccggcccccgccacacgctagtggaccccgaaggcgtctgggatgcgaacgggcctggaaccatagcgtcagggaggccggggtccccctgggcctgccagccccgggtgcgaggaggcgcgggggcagtgccagccgaagtctgccgttgcccaagaggcccaggcgtggcgctgcccctgagccggagcggacgcccgttgggcaggggtcctgggcccacccgggcaggacgcgtggaccgagtgaccgtggtttctgtgtggtgtcacctgccagacccgccgaagaagccacctctttggagggtgcgctctctggcacgcgccactcccacccatccgtgggccgccagcaccacgcgggccccccatccacatcgcggccaccacgtccctgggacacgccttgtcccccggtgtacgccgagaccaagcacttcctctactcctcaggcgacaaggagcagctgcggccctccttcctactcagctctctgaggcccagcctgactggcgctcggaggctcgtggagaccatctttctgggttccaggccctggatgccagggactccccgcaggttgccccgcctgccccagcgctactggcaaatgcggcccctgtttctggagctgcttgggaaccacgcgcagtgcccctacggggtgctcctcaagacgcactgcccgctgcgagctgcggtcaccccagcagccggtgtctgtgcccgggagaagccccagggctctgtggcggcccccgaggaggaggacacagacccccgtcgcctggtgcagctgctccgccagcacagcagcccctggcaggtgtacggcttcgtgcgggcctgcctgcgccggctggtgcccccaggcctctggggctccaggcacaacgaacgccgcttcctcaggaacaccaagaagttcatctccctggggaagcatgccaagctctcgctgcaggagctgacgtggaagatgagcgtgcgggactgcgcttggctgcgcaggagcccaggggttggctgtgttccggccgcagagcaccgtctgcgtgaggagatcctggccaagttcctgcactggctgatgagtgtgtacgtcgtcgagctgctcaggtctttcttttatgtcacggagaccacgtttcaaaagaacaggctctttttctaccggaagagtgtctggagcaagttgcaaagcattggaatcagacagcacttgaagagggtgcagctgcgggagctgtcggaagcagaggtcaggcagcatcgggaagccaggcccgccctgctgacgtccagactccgcttcatccccaagcctgacgggctgcggccgattgtgaacatggactacgtcgtgggagccagaacgttccgcagagaaaagagggccgagcgtctcacctcgagggtgaaggcactgttcagcgtgctcaactacgagcgggcgcggcgccccggcctcctgggcgcctctgtgctgggcctggacgatatccacagggcctggcgcaccttcgtgctgcgtgtgcgggcccaggacccgccgcctgagctgtactttgtcaaggtggatgtgacgggcgcgtacgacaccatcccccaggacaggctcacggaggtcatcgccagcatcatcaaaccccagaacacgtactgcgtgcgtcggtatgccgtggtccagaaggccgcccatgggcacgtccgcaaggccttcaagagccacgtctctaccttgacagacctccagccgtacatgcgacagttcgtggctcacctgcaggagaccagcccgctgagggatgccgtcgtcatcgagcagagctcctccctgaatgaggccagcagtggcctcttcgacgtcttcctacgcttcatgtgccaccacgccgtgcgcatcaggggcaagtcctacgtccagtgccaggggatcccgcagggctccatcctctccacgctgctctgcagcctgtgctacggcgacatggagaacaagctgtttgcggggattcggcgggacgggctgctcctgcgtttggtggatgatttcttgttggtgacacctcacctcacccacgcgaaaaccttcctcaggaccctggtccgaggtgtccctgagtatggctgcgtggtgaacttgcggaagacagtggtgaacttccctgtagaagacgaggccctgggtggcacggcttttgttcagatgccggcccacggcctattcccctggtgcggcctgctgctggatacccggaccctggaggtgcagagcgactactccagctatgcccggacctccatcagagccagtctcaccttcaaccgcggcttcaaggctgggaggaacatgcgtcgcaaactctttggggtcttgcggctgaagtgtcacagcctgtttctggatttgcaggtgaacagcctccagacggtgtgcaccaacatctacaagatcctcctgctgcaggcgtacaggtttcacgcatgtgtgctgcagctcccatttcatcagcaagtttggaagaaccccacatttttcctgcgcgtcatctctgacacggcctccctctgctactccatcctgaaagccaagaacgcagggatgtcgctgggggccaagggcgccgccggccctctgccctccgaggccgtgcagtggctgtgccaccaagcattcctgctcaagctgactcgacaccgtgtcacctacgtgccactcctggggtcactcaggacagcccagacgcagctgagtcggaagctcccggggacgacgctgactgccctggaggccgcagccaacccggcactgccctcagacttcaagaccatcctggactga

SEQ ID NO: 3 - DNA, 477 bp, Human papillomavirus type 16
  gene 1..477: note = HPV16 E6
  source 1..477: mol_type = other DNA
atgcaccaaaagagaactgcaatgtttcaggacccacaggagcgacccagaaagttaccacagttatgcacagagctgcaaacaactatacatgatataatattagaatgtgtgtactgcaagcaacagttactgcgacgtgaggtatatgactttgcttttcgggatttatgcatagtatatagagatgggaatccatatgctgtatgtgataaatgtttaaagttttattctaaaattagtgagtatagacattattgttatagtttgtatggaacaacattagaacagcaatacaacaaaccgttgtgtgatttgttaattaggtgtattaactgtcaaaagccactgtgtcctgaagaaaagcaaagacatctggacaaaaagcaaagattccataatataaggggtcggtggaccggtcgatgtatgtcttgttgcagatcatcaagaacacgtagagaaacccagctgtaa

SEQ ID NO: 4 - DNA, 297 bp, Human papillomavirus type 16
  gene 1..297: note = HPV 16 E7
  source 1..297: mol_type = other DNA
atgcatggagatacacctacattgcatgaatatatgttagatttgcaaccagagacaactgatctctactgttatgagcaattaaatgacagctcagaggaggaggatgaaatagatggtccagctggacaagcagaaccggacagagcccattacaatattgtaaccttttgttgcaagtgtgactctacgcttcggttgtgcgtacaaagcacacacgtagacattcgtactttggaagacctgttaatgggcacactaggaattgtgtgccccatctgttctcagaaaccataa

SEQ ID NO: 5 - DNA, 3396 bp, swine
  gene 1..3396: note = pigTERT
  source 1..3396: mol_type = genomic DNA
atgccgcgcgcgccccggtgccgggccgtgcgctccctgctccgggaccgctacaggcaggtgctgccgctggccaccttcgtgcggcgcctgggccctgagggccggcggcttgttcggcgcggggacccggcggcctaccgcgcgctggtggcgcagtgcctggtgtgcgtgccctgggacgcgcagccgcctcctgcctccccgtccttccgccaggtgtcctgcctgaaggagctggtggccagggtcgtgcagaggctctgcgagcgcggcgcgaggaacgtgctggcctttggcttcgcgctgctggacggggctcgcggcgggccgcccgtggccttcacgaccagcgtgcgcagctacctgcccaacaccgtgaccgacacactgcgcgggagcggcgcgtgggggctgctgctgcgccgcgtgggcgacgacgtgctcacccacctgttggcgcgctgcgcgctgtacctgctggtgcccccgagttgcgcctaccaggtgtgcgggccgccactctatgacctctacaccgcagcggaggctcggcccatgcgacacaagggccagaccccgactggcctcggactcacgcgccccgtttgcaatggggaagccgggcgaccccaggagcagagggcgcaaggtgtgaggcgacgtcggggcagagcggggggacatccacttccagccaagaggcccaggcacgtcccggagcctgaacagggtcccgaagggcaggcgtcccgggcccaccagggcagggcgcctgggccgagcgacagcgacccccccgtgatgacacctaccagagccgctgcgaaagccaagtctcgggagggtgaggcgcccggaacccggcacctttcccctcaagcaggcggtgcgcggggtacctgccccccatcctggtggcagccacacctccagggcaagcccagtcctcatgtgtgcgctgccgagaccaagcgcttcctctactgctcggggagcaaggaagggctgcgccgctcgttcctgctctgctccctgccgcccagcctggcgggggccgggaggctcgtggaggtcatctttctggcctcaaagcccgggcagccaggggcgcgccgcgtgcccgcacgctactggcggatgaggcccctgttccgggagctgcttaagaaccacgcgcggtgcccctacaaggcgcttctcagggcgcactgcccgttgcgggctgcggcgaccctctcggggtccggcggtcaggtgtgcgaccacaaagtgggccccctcgctccagagcggctggcagcggccgccgagggggactcggcctcgaggcgcctagtccagctgctccgccagcacagcagcccctggcaggtgtaccgcctcctgcgggcctgtcttcaccggctggtgcccccgggcctctggggctccccgcacaacaagcggcgctttctgaagaatgtgaagaagctcgtctccctggggaagcacgccaggctctcgctgcaggagctgatgtggaagatgaaagtgcaagactgcatctggctgcgccggagcccggacgctcgccatgtccaggccgccgagcaccgtctgagagaggccattctggccaagttcctgcgctggttgatgggcacgtacgtggtcgagctgctcaggtcgtttttttatgtcacggagaccacgtttcagaagaaccggctcttcttcttccggaagcgcatctggagccggctgcagagcgcaggcatcaggcaacacttagatcgtgtgcggcttcgagaactgtcggaagcagagatcaggcgacgccgggaggccaggcccgctgtactgacctccaagctccgcttcgtccccaaacccgacgggctgcggcccatcgtgaacatggcgaacgtcgtgcgagccaggacaggccccggagacaagaaggtccggcgtctcacggggcaggtcaagacgctgtttgctgtgctgaactacgagcgggcgcggcgcccgcgcctcctgggggcctccgtgctgggcgtgggtgacatccacagggcgtggcgggcctttgtgctgcccctgcgggcccaggacccggcccccccgctgtactttgtcaaggtggacgtgacgggggcctacgacgccctccctcaggacaggcttgctgaggtggtcgccaacgtgatccggccctacgagagcacgtactgcgtgcgccagtgcgccgtgctccggaggaccgcccgcgggcacgtgcgcaagtccttccaaacccacgtgtccaccttcgcagacctccagccttacatgagacagtttgtggcacacctgcaggcaaccggcccgctgagggacgccgtggtcatcgagcagagctgctctctgaacgaggccggcagccgtcccctggagcttttcctgagcctgctgcgaaaccacgtcatccggatcgggggcaggtcctacgtccagtgtcaggggatcccacagggctccattctgtccacgctgctctgcagcctgtgctacggggacatggaaaacagactgtccccggggatccagcgtgacggggtgctcctgcgcttggtggacgacttcctgctggtgacccctcacctgacacgagccaaagcctttctcaggaccctggtccgcggcgtgcccgagtacggctgcctggccaacttgcggaagacggccgtgaacttccctgtggaggacggcgcccggggcggcccggccccactgcagctgccggcacactgcctgttcccctggtgcgggctgctgctggacacccgcacgctggaggtgcactgcgactatgccagttacgcccggacctcgatcagagcgagtctcaccttcaaccagggcttcaagcccgggaggaacatgcgccgcaagctcttggcggtcttgcggctaaagtgccacgggatccttctggacctgcaggtgaacagtcttccgacggtgctcgccaacgtttacaagatcttcctgctgcaggcctacaggttccacgcgtgtgtgctgcagctgcccttccgtcagccgcttgcgaggaacccctcatttttcctccggcttgtctccgacaccgcgtcctgctgctactcgctcctgaaagccagaaacgcagggatgtccctgggagccaggggcgcctccggcccgtttccctctgaagccgcagagtggctctgcctccacgccttcctgctcaagctggttcgtcaccgcgttacctacagctgtcttctggggccgctccgggcagccagagagcgattgtgccagcggctccctggggccacactggccgccctcgaggccgccgccgacccagccctgactacagacttccggaccatcctggactga

SEQ ID NO: 6 - DNA, 981 bp, Homo sapiens
  gene 1..981: note = hbmi1
  source 1..981: mol_type = genomic DNA
atgcatcgaacaacgagaatcaagatcactgagctaaatccccacctgatgtgtgtgctttgtggagggtacttcattgatgccacaaccataatagaatgtctacattccttctgtaaaacgtgtattgttcgttacctggagaccagcaagtattgtcctatttgtgatgtccaagttcacaagaccagaccactactgaatataaggtcagataaaactctccaagatattgtatacaaattagttccagggcttttcaaaaatgaaatgaagagaagaagggatttttatgcagctcatccttctgctgatgctgccaatggctctaatgaagatagaggagaggttgcagatgaagataagagaattataactgatgatgagataataagcttatccattgaattctttgaccagaacagattggatcggaaagtaaacaaagacaaagagaaatctaaggaggaggtgaatgataaaagatacttacgatgcccagcagcaatgactgtgatgcacttaagaaagtttctcagaagtaaaatggacatacctaatactttccagattgatgtcatgtatgaggaggaacctttaaaggattattatacactaatggatattgcctacatttatacctggagaaggaatggtccacttccattgaaatacagagttcgacctacttgtaaaagaatgaagatcagtcaccagagagatggactgacaaatgctggagaactggaaagtgactctgggagtgacaaggccaacagcccagcaggaggtattccctccacctcttcttgtttgcctagccccagtactccagtgcagtctcctcatccacagtttcctcacatttccagtactatgaatggaaccagcaacagccccagcggtaaccaccaatcttcttttgccaatagacctcgaaaatcatcagtaaatgggtcatcagcaacttcttctggttga

SEQ ID NO: 7 - DNA, 20 bp, synthetic construct
  misc_feature 1..20: note = a primer for real-time PCR
  source 1..20: mol_type = other DNA
ggcactgccctcagacttca

SEQ ID NO: 8 - DNA, 20 bp, synthetic construct
  misc_feature 1..20: note = a primer for real-time PCR
  source 1..20: mol_type = other DNA
ctgctaaagcgcatgctcca

SEQ ID NO: 9 - DNA, 19 bp, synthetic construct
  misc_feature 1..19: note = a primer for real-time PCR
  source 1..19: mol_type = other DNA
ctgcggcatccacgaacta

SEQ ID NO: 10 - DNA, 19 bp, synthetic construct
  misc_feature 1..19: note = a primer for real-time PCR
  source 1..19: mol_type = other DNA
acagcaccgtgttggcgta

SEQ ID NO: 11 - DNA, 24 bp, synthetic construct
  misc_feature 1..24: note = a primer for real-time PCR
  source 1..24: mol_type = other DNA
ttggtcaagcagcataatccaaag

SEQ ID NO: 12 - DNA, 23 bp, synthetic construct
  misc_feature 1..23: note = a primer for real-time PCR
  source 1..23: mol_type = other DNA
gtcaagggcatagcctaccacaa

SEQ ID NO: 13 - DNA, 22 bp, synthetic construct
  misc_feature 1..22: note = a primer for real-time PCR
  source 1..22: mol_type = other DNA
gcactgccctcagacttcaaga

SEQ ID NO: 14 - DNA, 20 bp, synthetic construct
  misc_feature 1..20: note = a primer for real-time PCR
  source 1..20: mol_type = other DNA
gcgggactatggttgctgac

SEQ ID NO: 15 - DNA, 19 bp, synthetic construct
  misc_feature 1..19: note = a primer for real-time PCR
  source 1..19: mol_type = other DNA
tggcacccagcacaatgaa

SEQ ID NO: 16 - DNA, 26 bp, synthetic construct
  misc_feature 1..26: note = a primer for real-time PCR
  source 1..26: mol_type = other DNA
ctaagtcatagtccgcctagaagcca

SEQ ID NO: 17 - DNA, 20 bp, synthetic construct
  misc_feature 1..20: note = a primer for real-time PCR
  source 1..20: mol_type = other DNA
tgatttcgagcgtggcagag

SEQ ID NO: 18 - DNA, 20 bp, synthetic construct
  misc_feature 1..20: note = a primer for real-time PCR
  source 1..20: mol_type = other DNA
acatttggcggccacacata

SEQ ID NO: 19 - DNA, 19 bp, synthetic construct
  misc_feature 1..19: note = a primer for real-time PCR
  source 1..19: mol_type = other DNA
tatggcccagaccctcaca

SEQ ID NO: 20 - DNA, 24 bp, synthetic construct
  misc_feature 1..24: note = a primer for real-time PCR
  source 1..24: mol_type = other DNA
ggagtagacaaggtacaacccatc

SEQ ID NO: 21 - DNA, 22 bp, synthetic construct
  misc_feature 1..22: note = a primer for real-time PCR
  source 1..22: mol_type = other DNA
cggcacagtcattgaaagccta

SEQ ID NO: 22 - DNA, 21 bp, synthetic construct
  misc_feature 1..21: note = a primer for real-time PCR
  source 1..21: mol_type = other DNA
gttgctgatggcctgattgtc

SEQ ID NO: 23 - DNA, 19 bp, synthetic construct
  misc_feature 1..19: note = a primer for real-time PCR
  source 1..19: mol_type = other DNA
ctgatcaggacgcgcaaac

SEQ ID NO: 24 - DNA, 20 bp, synthetic construct
  misc_feature 1..20: note = a primer for real-time PCR
  source 1..20: mol_type = other DNA
tcgctgctgccttcactgta

SEQ ID NO: 25 - DNA, 25 bp, synthetic construct
  misc_feature 1..25: note = a primer for real-time PCR
  source 1..25: mol_type = other DNA
ttgttgttggatatgcccttgacta

SEQ ID NO: 26 - DNA, 21 bp, synthetic construct
  misc_feature 1..21: note = a primer for real-time PCR
  source 1..21: mol_type = other DNA
aggcagatggccacaggacta